European Patent Application EP 4 714 975 A1, published March 25, 2026. Title: 结合LILRB4和CD3的抗体及其用途. Applicant: 南京维立志博生物科技有限公司. The sequence listing filed with the application follows.

SEQUENCE LISTING (87 sequences)

SEQ ID NO: 1 - protein, 455 aa, artificial sequence
EVQLVESGGGLVQPGGSLKLSCAASGFTFSTYAMNWVRQAPGKGLEWVGRIRSKYNNYATYYADSVKDRFTISRDDSKNTLYLQMNSLKTEDTAVYYCTRHGNFGNSYVSWFAYWGQGTTVTVSSASTKGPSVFPLAPSSKSTSGGTAALGCLVKDYFPEPVTVSWNSGALTSGVHTFPAVLQSSGLYSLSSVVTVPSSSLGTQTYICNVNHKPSNTKVDKKVEPKSCDKTHTCPPCPAPEAAGGPSVFLFPPKPKDTLMISRTPEVTCVVVAVSHEDPEVKFNWYVDGVEVHNAKTKPREEQYNSTYRVVSVLTVLHQDWLNGKEYKCKVSNKALAAPIEKTISKAKGQPREPQVYTLPPSRDELTKNQVSLTCLVKGFYPSDIAVEWESNGQPENNYKTTPPVLDSDGSFFLYSKLTVDKSRWQQGNVFSCSVMHEALHNHYTQKSLSLSPGK

SEQ ID NO: 2 - protein, 214 aa, artificial sequence
QAVVTQEPSLTVSPGGTVTLTCRSSTGAVTTSNYANWVQQKPGQAPRGLIGGTNKRAPGVPARFSGSLLGGKAALTLSGAQPEDEAEYFCALWYSNLWVFGGGTKLTVLGQPKAAPSVTLFPPSSEELQANKATLVCLISDFYPGAVTVAWKADSSPVKAGVETTTPSKQSNNKYAASSYLSLTPEQWKSHRSYSCQVTHEGSTVEKTVAPTEC

SEQ ID NO: 3 - protein, 125 aa, artificial sequence
EVQLVESGGGLVQPGGSLKLSCAASGFTFSTYAMNWVRQAPGKGLEWVGRIRSKYNNYATYYADSVKDRFTISRDDSKNTLYLQMNSLKTEDTAVYYCTRHGNFGNSYVSWFAYWGQGTTVTVSS

SEQ ID NO: 4 - protein, 109 aa, artificial sequence
QAVVTQEPSLTVSPGGTVTLTCRSSTGAVTTSNYANWVQQKPGQAPRGLIGGTNKRAPGVPARFSGSLLGGKAALTLSGAQPEDEAEYFCALWYSNLWVFGGGTKLTVL

SEQ ID NO: 5 - protein, 5 aa, artificial sequence
TYAMN

SEQ ID NO: 6 - protein, 19 aa, artificial sequence
RIRSKYNNYATYYADSVKD

SEQ ID NO: 7 - protein, 14 aa, artificial sequence
HGNFGNSYVSWFAY

SEQ ID NO: 8 - protein, 14 aa, artificial sequence
RSSTGAVTTSNYAN

SEQ ID NO: 9 - protein, 7 aa, artificial sequence
GTNKRAP

SEQ ID NO: 10 - protein, 9 aa, artificial sequence
ALWYSNLWV

SEQ ID NO: 11 - protein, 119 aa, artificial sequence
QVQLVESGGGLVQPGGSLRLSCAASGFTFSSYTMSWVRQAPGKGLEWISDINNDGGKTYYAFSVEGRFTISRDNAKNTLYLQMNSLKPEDTAVYYCVRDHQYTSRNGDRGQGTQVTVSS

SEQ ID NO: 12 - protein, 8 aa, artificial sequence
GFTFSSYT

SEQ ID NO: 13 - protein, 8 aa, artificial sequence
INNDGGKT

SEQ ID NO: 14 - protein, 12 aa, artificial sequence
VRDHQYTSRNGD

SEQ ID NO: 15 - protein, 351 aa, artificial sequence
QVQLVESGGGLVQPGGSLRLSCAASGFTFSSYTMSWVRQAPGKGLEWISDINNDGGKTYYAFSVEGRFTISRDNAKNTLYLQMNSLKPEDTAVYYCVRDHQYTSRNGDRGQGTQVTVSSEPKSSDKTHTCPPCPAPELLGGPSVFLFPPKPKDTLMISRTPEVTCVVVDVSHEDPEVKFNWYVDGVEVHNAKTKPREEQYNSTYRVVSVLTVLHQDWLNGKEYKCKVSNKALPAPIEKTISKAKGQPREPQVYTLPPSRDELTKNQVSLTCLVKGFYPSDIAVEWESNGQPENNYKTTPPVLDSDGSFFLYSKLTVDKSRWQQGNVFSCSVMHEALHNHYTQKSLSLSPGK

SEQ ID NO: 16 - protein, 121 aa, artificial sequence
EVQLVESGGGLVQAGGSLRLSCAASESIFSSNVMGWYRQSPGHQRELVAAVGINGLTKIGDSVKGRFTISRDNAKNTVYLQMNSLKVEDTAVYYCAAGAYVRFLQNSPDYWGQGTQVTVSS

SEQ ID NO: 17 - protein, 8 aa, artificial sequence
ESIFSSNV

SEQ ID NO: 18 - protein, 7 aa, artificial sequence
VGINGLT

SEQ ID NO: 19 - protein, 15 aa, artificial sequence
AAGAYVRFLQNSPDY

SEQ ID NO: 20 - protein, 353 aa, artificial sequence
EVQLVESGGGLVQAGGSLRLSCAASESIFSSNVMGWYRQSPGHQRELVAAVGINGLTKIGDSVKGRFTISRDNAKNTVYLQMNSLKVEDTAVYYCAAGAYVRFLQNSPDYWGQGTQVTVSSEPKSSDKTHTCPPCPAPELLGGPSVFLFPPKPKDTLMISRTPEVTCVVVDVSHEDPEVKFNWYVDGVEVHNAKTKPREEQYNSTYRVVSVLTVLHQDWLNGKEYKCKVSNKALPAPIEKTISKAKGQPREPQVYTLPPSRDELTKNQVSLTCLVKGFYPSDIAVEWESNGQPENNYKTTPPVLDSDGSFFLYSKLTVDKSRWQQGNVFSCSVMHEALHNHYTQKSLSLSPGK

SEQ ID NO: 21 - protein, 121 aa, artificial sequence
EVQVVESGGGLVQAGGSLRLSCAASETIFSSNVMGWYRQAHGKQRELVAATGINGVTKYADSVKGRFTISRDNAKNTVYLQMNSLNVEDTAVYYCAAGVWRNFVMRSPDYWGQGTQVTVSS

SEQ ID NO: 22 - protein, 7 aa, artificial sequence
TGINGVT

SEQ ID NO: 23 - protein, 15 aa, artificial sequence
AAGVWRNFVMRSPDY

SEQ ID NO: 24 - protein, 353 aa, artificial sequence
EVQVVESGGGLVQAGGSLRLSCAASETIFSSNVMGWYRQAHGKQRELVAATGINGVTKYADSVKGRFTISRDNAKNTVYLQMNSLNVEDTAVYYCAAGVWRNFVMRSPDYWGQGTQVTVSSEPKSSDKTHTCPPCPAPELLGGPSVFLFPPKPKDTLMISRTPEVTCVVVDVSHEDPEVKFNWYVDGVEVHNAKTKPREEQYNSTYRVVSVLTVLHQDWLNGKEYKCKVSNKALPAPIEKTISKAKGQPREPQVYTLPPSRDELTKNQVSLTCLVKGFYPSDIAVEWESNGQPENNYKTTPPVLDSDGSFFLYSKLTVDKSRWQQGNVFSCSVMHEALHNHYTQKSLSLSPGK

SEQ ID NO: 25 - protein, 123 aa, artificial sequence
EVQVVESGGGSVQTGGSLTLSCAASGRTFRSNGMGWFRQAPGKEREFVAAIRWSGRRTTYTDSVKGRFTISSDSAKNTVYLQMSSLKPEDTAVYYCAVDLLPPYGALDKYDYWGQGTQVTVSS

SEQ ID NO: 26 - protein, 8 aa, artificial sequence
GRTFRSNG

SEQ ID NO: 27 - protein, 8 aa, artificial sequence
IRWSGRRT

SEQ ID NO: 28 - protein, 16 aa, artificial sequence
AVDLLPPYGALDKYDY

SEQ ID NO: 29 - protein, 355 aa, artificial sequence
EVQVVESGGGSVQTGGSLTLSCAASGRTFRSNGMGWFRQAPGKEREFVAAIRWSGRRTTYTDSVKGRFTISSDSAKNTVYLQMSSLKPEDTAVYYCAVDLLPPYGALDKYDYWGQGTQVTVSSEPKSSDKTHTCPPCPAPELLGGPSVFLFPPKPKDTLMISRTPEVTCVVVDVSHEDPEVKFNWYVDGVEVHNAKTKPREEQYNSTYRVVSVLTVLHQDWLNGKEYKCKVSNKALPAPIEKTISKAKGQPREPQVYTLPPSRDELTKNQVSLTCLVKGFYPSDIAVEWESNGQPENNYKTTPPVLDSDGSFFLYSKLTVDKSRWQQGNVFSCSVMHEALHNHYTQKSLSLSPGK

SEQ ID NO: 30 - protein, 121 aa, artificial sequence
EVQLVESGGGLVQPGGSLRLSCAASESIFSSNVMGWYRQAPGKQRELVAAVGINGLTKIGDSVKGRFTISRDNAKNSVYLQMNSLRAEDTAVYYCAAGAYVRFLQNSPDYWGQGTQVTVSS

SEQ ID NO: 31 - protein, 353 aa, artificial sequence
EVQLVESGGGLVQPGGSLRLSCAASESIFSSNVMGWYRQAPGKQRELVAAVGINGLTKIGDSVKGRFTISRDNAKNSVYLQMNSLRAEDTAVYYCAAGAYVRFLQNSPDYWGQGTQVTVSSEPKSSDKTHTCPPCPAPELLGGPSVFLFPPKPKDTLMISRTPEVTCVVVDVSHEDPEVKFNWYVDGVEVHNAKTKPREEQYNSTYRVVSVLTVLHQDWLNGKEYKCKVSNKALPAPIEKTISKAKGQPREPQVYTLPPSRDELTKNQVSLTCLVKGFYPSDIAVEWESNGQPENNYKTTPPVLDSDGSFFLYSKLTVDKSRWQQGNVFSCSVMHEALHNHYTQKSLSLSPGK

SEQ ID NO: 32 - protein, 121 aa, artificial sequence
EVQLVESGGGLVQPGGSLRLSCAASESIFSSNVMGWYRQAPGKQRELVAAVGINRLTKIGDSVKGRFTISRDNAKNSVYLQMNSLRAEDTAVYYCAAGAYVRFLQQSPDYWGQGTQVTVSS

SEQ ID NO: 33 - protein, 7 aa, artificial sequence
VGINRLT

SEQ ID NO: 34 - protein, 15 aa, artificial sequence
AAGAYVRFLQQSPDY

SEQ ID NO: 35 - protein, 353 aa, artificial sequence
EVQLVESGGGLVQPGGSLRLSCAASESIFSSNVMGWYRQAPGKQRELVAAVGINRLTKIGDSVKGRFTISRDNAKNSVYLQMNSLRAEDTAVYYCAAGAYVRFLQQSPDYWGQGTQVTVSSEPKSSDKTHTCPPCPAPELLGGPSVFLFPPKPKDTLMISRTPEVTCVVVDVSHEDPEVKFNWYVDGVEVHNAKTKPREEQYNSTYRVVSVLTVLHQDWLNGKEYKCKVSNKALPAPIEKTISKAKGQPREPQVYTLPPSRDELTKNQVSLTCLVKGFYPSDIAVEWESNGQPENNYKTTPPVLDSDGSFFLYSKLTVDKSRWQQGNVFSCSVMHEALHNHYTQKSLSLSPGK

SEQ ID NO: 36 - protein, 121 aa, artificial sequence
EVQLVESGGGLVQPGGSLRLSCAASESIFSSNVMGWYRQAPGKQRELVAAVGIQGLTKIGDSVKGRFTISRDNAKNSVYLQMNSLRAEDTAVYYCAAGAYVRFLQQSPDYWGQGTQVTVSS

SEQ ID NO: 37 - protein, 7 aa, artificial sequence
VGIQGLT

SEQ ID NO: 38 - protein, 353 aa, artificial sequence
EVQLVESGGGLVQPGGSLRLSCAASESIFSSNVMGWYRQAPGKQRELVAAVGIQGLTKIGDSVKGRFTISRDNAKNSVYLQMNSLRAEDTAVYYCAAGAYVRFLQQSPDYWGQGTQVTVSSEPKSSDKTHTCPPCPAPELLGGPSVFLFPPKPKDTLMISRTPEVTCVVVDVSHEDPEVKFNWYVDGVEVHNAKTKPREEQYNSTYRVVSVLTVLHQDWLNGKEYKCKVSNKALPAPIEKTISKAKGQPREPQVYTLPPSRDELTKNQVSLTCLVKGFYPSDIAVEWESNGQPENNYKTTPPVLDSDGSFFLYSKLTVDKSRWQQGNVFSCSVMHEALHNHYTQKSLSLSPGK

SEQ ID NO: 39 - protein, 121 aa, artificial sequence
EVQLVESGGGLVQPGGSLRLSCAASESIFSSNVMGWYRQAPGKQRELVAAVGINRLTKIGDSVKGRFTISRDNAKNSVYLQMNSLRAEDTAVYYCAAGAYVRFLQYSPDYWGQGTQVTVSS

SEQ ID NO: 40 - protein, 15 aa, artificial sequence
AAGAYVRFLQYSPDY

SEQ ID NO: 41 - protein, 353 aa, artificial sequence
EVQLVESGGGLVQPGGSLRLSCAASESIFSSNVMGWYRQAPGKQRELVAAVGINRLTKIGDSVKGRFTISRDNAKNSVYLQMNSLRAEDTAVYYCAAGAYVRFLQYSPDYWGQGTQVTVSSEPKSSDKTHTCPPCPAPELLGGPSVFLFPPKPKDTLMISRTPEVTCVVVDVSHEDPEVKFNWYVDGVEVHNAKTKPREEQYNSTYRVVSVLTVLHQDWLNGKEYKCKVSNKALPAPIEKTISKAKGQPREPQVYTLPPSRDELTKNQVSLTCLVKGFYPSDIAVEWESNGQPENNYKTTPPVLDSDGSFFLYSKLTVDKSRWQQGNVFSCSVMHEALHNHYTQKSLSLSPGK

SEQ ID NO: 42 - protein, 121 aa, artificial sequence
EVQLVESGGGLVQPGGSLRLSCAASESIFSSNVMGWYRQAPGKQRELVAAVGIQGLTKIGDSVKGRFTISRDNAKNSVYLQMNSLRAEDTAVYYCAAGAYVRFLQYSPDYWGQGTQVTVSS

SEQ ID NO: 43 - protein, 353 aa, artificial sequence
EVQLVESGGGLVQPGGSLRLSCAASESIFSSNVMGWYRQAPGKQRELVAAVGIQGLTKIGDSVKGRFTISRDNAKNSVYLQMNSLRAEDTAVYYCAAGAYVRFLQYSPDYWGQGTQVTVSSEPKSSDKTHTCPPCPAPELLGGPSVFLFPPKPKDTLMISRTPEVTCVVVDVSHEDPEVKFNWYVDGVEVHNAKTKPREEQYNSTYRVVSVLTVLHQDWLNGKEYKCKVSNKALPAPIEKTISKAKGQPREPQVYTLPPSRDELTKNQVSLTCLVKGFYPSDIAVEWESNGQPENNYKTTPPVLDSDGSFFLYSKLTVDKSRWQQGNVFSCSVMHEALHNHYTQKSLSLSPGK

SEQ ID NO: 44 - protein, 455 aa, artificial sequence
EVQLVESGGGLVQPGGSLKLSCAASGFTFSTYAMNWVRQAPGKGLEWVGRIRSKYNNYATYYADSVKDRFTISRDDSKNTLYLQMNSLKTEDTAVYYCTRHGNFGNSYVSWFAYWGQGTTVTVSSASTKGPSVFPLAPSSKSTSGGTAALGCLVKDYFPEPVTVSWNSGALTSGVHTFPAVLQSSGLYSLSSVVTVPSSSLGTQTYICNVNHKPSNTKVDKKVEPKSCDKTHTCPPCPAPEAAGGPSVFLFPPKPKDTLMISRTPEVTCVVVAVSHEDPEVKFNWYVDGVEVHNAKTKPREEQYNSTYRVVSVLTVLHQDWLNGKEYKCKVSNKALAAPIEKTISKAKGQPREPQVYTLPPCRDELTKNQVSLWCLVKGFYPSDIAVEWESNGQPENNYKTTPPVLDSDGSFFLYSKLTVDKSRWQQGNVFSCSVMHEALHNHYTQKSLSLSPGK

SEQ ID NO: 45 - protein, 353 aa, artificial sequence
EVQLVESGGGLVQPGGSLRLSCAASESIFSSNVMGWYRQAPGKQRELVAAVGIQGLTKIGDSVKGRFTISRDNAKNSVYLQMNSLRAEDTAVYYCAAGAYVRFLQQSPDYWGQGTQVTVSSEPKSSDKTHTCPPCPAPEAAGGPSVFLFPPKPKDTLMISRTPEVTCVVVAVSHEDPEVKFNWYVDGVEVHNAKTKPREEQYNSTYRVVSVLTVLHQDWLNGKEYKCKVSNKALAAPIEKTISKAKGQPREPQVCTLPPSRDELTKNQVSLSCAVKGFYPSDIAVEWESNGQPENNYKTTPPVLDSDGSFFLVSKLTVDKSRWQQGNVFSCSVMHEALHNHYTQKSLSLSPGK

SEQ ID NO: 46 - protein, 581 aa, artificial sequence
EVQLVESGGGLVQPGGSLRLSCAASESIFSSNVMGWYRQAPGKQRELVAAVGIQGLTKIGDSVKGRFTISRDNAKNSVYLQMNSLRAEDTAVYYCAAGAYVRFLQQSPDYWGQGTQVTVSSGGGGSEVQLVESGGGLVQPGGSLKLSCAASGFTFSTYAMNWVRQAPGKGLEWVGRIRSKYNNYATYYADSVKDRFTISRDDSKNTLYLQMNSLKTEDTAVYYCTRHGNFGNSYVSWFAYWGQGTTVTVSSASTKGPSVFPLAPSSKSTSGGTAALGCLVKDYFPEPVTVSWNSGALTSGVHTFPAVLQSSGLYSLSSVVTVPSSSLGTQTYICNVNHKPSNTKVDKKVEPKSCDKTHTCPPCPAPEAAGGPSVFLFPPKPKDTLMISRTPEVTCVVVAVSHEDPEVKFNWYVDGVEVHNAKTKPREEQYNSTYRVVSVLTVLHQDWLNGKEYKCKVSNKALAAPIEKTISKAKGQPREPQVYTLPPCRDELTKNQVSLWCLVKGFYPSDIAVEWESNGQPENNYKTTPPVLDSDGSFFLYSKLTVDKSRWQQGNVFSCSVMHEALHNHYTQKSLSLSPGK

SEQ ID NO: 47 - protein, 227 aa, artificial sequence
DKTHTCPPCPAPEAAGGPSVFLFPPKPKDTLMISRTPEVTCVVVAVSHEDPEVKFNWYVDGVEVHNAKTKPREEQYNSTYRVVSVLTVLHQDWLNGKEYKCKVSNKALAAPIEKTISKAKGQPREPQVCTLPPSRDELTKNQVSLSCAVKGFYPSDIAVEWESNGQPENNYKTTPPVLDSDGSFFLVSKLTVDKSRWQQGNVFSCSVMHEALHNHYTQKSLSLSPGK

SEQ ID NO: 48 - protein, 232 aa, artificial sequence
EPKSSDKTHTCPPCPAPEAAGGPSVFLFPPKPKDTLMISRTPEVTCVVVAVSHEDPEVKFNWYVDGVEVHNAKTKPREEQYNSTYRVVSVLTVLHQDWLNGKEYKCKVSNKALAAPIEKTISKAKGQPREPQVCTLPPSRDELTKNQVSLSCAVKGFYPSDIAVEWESNGQPENNYKTTPPVLDSDGSFFLVSKLTVDKSRWQQGNVFSCSVMHEALHNHYTQKSLSLSPGK

SEQ ID NO: 49 - protein, 232 aa, artificial sequence
EPKSCDKTHTCPPCPAPEAAGGPSVFLFPPKPKDTLMISRTPEVTCVVVAVSHEDPEVKFNWYVDGVEVHNAKTKPREEQYNSTYRVVSVLTVLHQDWLNGKEYKCKVSNKALAAPIEKTISKAKGQPREPQVYTLPPCRDELTKNQVSLWCLVKGFYPSDIAVEWESNGQPENNYKTTPPVLDSDGSFFLYSKLTVDKSRWQQGNVFSCSVMHEALHNHYTQKSLSLSPGK

SEQ ID NO: 50 - protein, 227 aa, artificial sequence
DKTHTCPPCPAPEAAGGPSVFLFPPKPKDTLMISRTPEVTCVVVAVSHEDPEVKFNWYVDGVEVHNAKTKPREEQYNSTYRVVSVLTVLHQDWLNGKEYKCKVSNKALAAPIEKTISKAKGQPREPQVYTLPPCRDELTKNQVSLWCLVKGFYPSDIAVEWESNGQPENNYKTTPPVLDSDGSFFLYSKLTVDKSRWQQGNVFSCSVMHEALHNHYTQKSLSLSPGK

SEQ ID NO: 51 - protein, 98 aa, artificial sequence
ASTKGPSVFPLAPSSKSTSGGTAALGCLVKDYFPEPVTVSWNSGALTSGVHTFPAVLQSSGLYSLSSVVTVPSSSLGTQTYICNVNHKPSNTKVDKKV

SEQ ID NO: 52 - protein, 332 aa, artificial sequence
ASTKGPSVFPLAPSSKSTSGGTAALGCLVKDYFPEPVTVSWNSGALTSGVHTFPAVLQSSGLYSLSSVVTVPSSSLGTQTYICNVNHKPSNTKVDKKVEPKSCDKTHTCPPCPAPEAAGGPSVFLFPPKPKDTLMISRTPEVTCVVVAVSHEDPEVKFNWYVDGVEVHNAKTKPREEQYNSTYRVVSVLTVLHQDWLNGKEYKCKVSNKALAAPIEKTISKAKGQPREPQVYTLPPSRDELTKNQVSLTCLVKGFYPSDIAVEWESNGQPENNYKTTPPVLDSDGSFFLYSKLTVDKSRWQQGNVFSCSVMHEALHNHYTQKSLSLSPGKFC

SEQ ID NO: 53 - protein, 227 aa, artificial sequence
DKTHTCPPCPAPEAAGGPSVFLFPPKPKDTLMISRTPEVTCVVVAVSHEDPEVKFNWYVDGVEVHNAKTKPREEQYNSTYRVVSVLTVLHQDWLNGKEYKCKVSNKALAAPIEKTISKAKGQPREPQVYTLPPSRDELTKNQVSLTCLVKGFYPSDIAVEWESNGQPENNYKTTPPVLDSDGSFFLYSKLTVDKSRWQQGNVFSCSVMHEALHNHYTQKSLSLSPGK

SEQ ID NO: 54 - protein, 232 aa, artificial sequence
EPKSSDKTHTCPPCPAPEAAGGPSVFLFPPKPKDTLMISRTPEVTCVVVAVSHEDPEVKFNWYVDGVEVHNAKTKPREEQYNSTYRVVSVLTVLHQDWLNGKEYKCKVSNKALAAPIEKTISKAKGQPREPQVYTLPPSRDELTKNQVSLTCLVKGFYPSDIAVEWESNGQPENNYKTTPPVLDSDGSFFLYSKLTVDKSRWQQGNVFSCSVMHEALHNHYTQKSLSLSPGK

SEQ ID NO: 55 - protein, 227 aa, artificial sequence
DKTHTCPPCPAPELLGGPSVFLFPPKPKDTLMISRTPEVTCVVVDVSHEDPEVKFNWYVDGVEVHNAKTKPREEQYNSTYRVVSVLTVLHQDWLNGKEYKCKVSNKALPAPIEKTISKAKGQPREPQVYTLPPSRDELTKNQVSLTCLVKGFYPSDIAVEWESNGQPENNYKTTPPVLDSDGSFFLYSKLTVDKSRWQQGNVFSCSVMHEALHNHYTQKSLSLSPGK

SEQ ID NO: 56 - protein, 105 aa, artificial sequence
GQPKAAPSVTLFPPSSEELQANKATLVCLISDFYPGAVTVAWKADSSPVKAGVETTTPSKQSNNKYAASSYLSLTPEQWKSHRSYSCQVTHEGSTVEKTVAPTEC

SEQ ID NO: 57 - protein, 330 aa, artificial sequence [sequence omitted]

SEQ ID NO: 58 - protein, 107 aa, artificial sequence [sequence omitted]

SEQ ID NO: 59 - protein, 5 aa, artificial sequence
EPKSS

SEQ ID NO: 60 - protein, 5 aa, artificial sequence
GGGGS

SEQ ID NO: 61 - protein, 450 aa, artificial sequence
EVQLVESGGGLVQPGGSLRLSCAASGFSLSSSYWISWVRQAPGKGLEWIGSIDSGSVGITYYATWVKGRFTISRDNSKNTLYLQMNSLRAEDTAVYYCARHGDNWALDLWGQGTLVTVSSASTKGPSVFPLAPSSKSTSGGTAALGCLVKDYFPEPVTVSWNSGALTSGVHTFPAVLQSSGLYSLSSVVTVPSSSLGTQTYICNVNHKPSNTKVDKKVEPKSCDKTHTCPPCPAPELLGGPSVFLFPPKPKDTLMISRTPEVTCVVVDVSHEDPEVKFNWYVDGVEVHNAKTKPREEQYNSTYRVVSVLTVLHQDWLNGKEYKCKVSNKALPAPIEKTISKAKGQPREPQVYTLPPSRDELTKNQVSLTCLVKGFYPSDIAVEWESNGQPENNYKTTPPVLDSDGSFFLYSKLTVDKSRWQQGNVFSCSVMHEALHNHYTQKSLSLSPGK

SEQ ID NO: 62 - protein, 217 aa, artificial sequence
DLVMTQSPSTLSASVGDRVTITCQASQSINSWLAWYQQKPGKPPKLLIYKASTLASGVSSRFSGSGSGTEFTLTISSLQPDDVATYYCQHGYIRGDLDNVFGGGTKVEIKRTVAAPSVFIFPPSDEQLKSGTASVVCLLNNFYPREAKVQWKVDNALQSGNSQESVTEQDSKDSTYSLSSTLTLSKADYEKHKVYACEVTHQGLSSPVTKSFNRGEC

SEQ ID NO: 63 - protein, 455 aa, artificial sequence
EVQLLESGGGLVQPGGSLRLSCAASGFTFSTYAMNWVRQAPGKGLEWVSRIRSKYNNYATYYADSVKGRFTISRDDSKNTLYLQMNSLRAEDTAVYYCVRHGNFGNSYVSWFAYWGQGTLVTVSSASTKGPSVFPLAPSSKSTSGGTAALGCLVKDYFPEPVTVSWNSGALTSGVHTFPAVLQSSGLYSLSSVVTVPSSSLGTQTYICNVNHKPSNTKVDKKVEPKSCDKTHTCPPCPAPEAAGGPSVFLFPPKPKDTLMISRTPEVTCVVVAVSHEDPEVKFNWYVDGVEVHNAKTKPREEQYNSTYRVVSVLTVLHQDWLNGKEYKCKVSNKALAAPIEKTISKAKGQPREPQVYTLPPSRDELTKNQVSLTCLVKGFYPSDIAVEWESNGQPENNYKTTPPVLDSDGSFFLYSKLTVDKSRWQQGNVFSCSVMHEALHNHYTQKSLSLSPGK

SEQ ID NO: 64 - protein, 214 aa, artificial sequence
QAVVTQEPSLTVSPGGTVTLTCGSSTGAVTTSNYANWVQEKPGQAFRGLIGGTNKRAPGTPARFSGSLLGGKAALTLSGAQPEDEAEYYCALWYSNLWVFGGGTKLTVLGQPKAAPSVTLFPPSSEELQANKATLVCLISDFYPGAVTVAWKADSSPVKAGVETTTPSKQSNNKYAASSYLSLTPEQWKSHRSYSCQVTHEGSTVEKTVAPTEC

SEQ ID NO: 65 - protein, 280 aa, artificial sequence
MIPTFTALLCLGLSLGPRTHMQAGPLPKPTLWAEPGSVISWGNSVTIWCQGTLEAREYRLDKEESPAPWDRQNPLEPKNKARFSIPSMTEDYAGRYRCYYRSPVGWSQPSDPLELVMTGAYSKPTLSALPSPLVTSGKSVTLLCQSRSPMDTFLLIKERAAHPLLHLRSEHGAQQHQAEFPMSPVTSVHGGTYRCFSSHGFSHYLLSHPSDPLELIVSGSLEDPRPSPTRSVSTAAGPEDQPLMPTGSVPHSGLRRHWEVLIGVLVVSILLLSLLLFLLL

SEQ ID NO: 66 - protein, 280 aa, artificial sequence
MTPPLTVLFCLGLSLGPRTCVQAGPLPKPTVWAEPGSVISWGSPVTIWCQGTLDAQEYHLDKEGSPAPWDTQNPLEPRNKAKFSIPSMTQHYAGRYRCYYHSHPDWSEDSDPLDLVMTGAYSKPILSVLPSPLVTSGESVTLLCQSQSPMDTFLLFKEGAAHPLPRLRSQHGAQLHWAEFPMGPVTSVHGGTYRCISSRSFSHYLLSRPSDPVELTVLGSLESPSPSPTRSISAAAGPEDQSLMPTGSDPQSGLRRHWEVLIGVLVVSILLLSLVFFLLL

SEQ ID NO: 67 - protein, 5 aa, artificial sequence
EPKSC

SEQ ID NO: 68 - protein, 232 aa, artificial sequence
EPKSCDKTHTCPPCPAPELLGGPSVFLFPPKPKDTLMISRTPEVTCVVVDVSHEDPEVKFNWYVDGVEVHNAKTKPREEQYNSTYRVVSVLTVLHQDWLNGKEYKCKVSNKALPAPIEKTISKAKGQPREPQVYTLPPSRDELTKNQVSLTCLVKGFYPSDIAVEWESNGQPENNYKTTPPVLDSDGSFFLYSKLTVDKSRWQQGNVFSCSVMHEALHNHYTQKSLSLSPGK

SEQ ID NO: 69 - protein, 250 aa, artificial sequence
EVQLVESGGGLVQPGGSLKLSCAASGFTFSTYAMNWVRQAPGKGLEWVGRIRSKYNNYATYYADSVKDRFTISRDDSKNTLYLQMNSLKTEDTAVYYCTRHGNFGNSYVSWFAYWGQGTTVTVSSGGGGSGGGGSGGGGSQAVVTQEPSLTVSPGGTVTLTCRSSTGAVTTSNYANWVQQKPGQAPRGLIGGTNKRAPGVPARFSGSLLGGKAALTLSGAQPEDEAEYFCALWYSNLWVFGGGTKLTVLG

SEQ ID NO: 70 - protein, 15 aa, artificial sequence
GGGGSGGGGSGGGGS

SEQ ID NO: 71 - protein, 477 aa, artificial sequence
EVQLVESGGGLVQPGGSLKLSCAASGFTFSTYAMNWVRQAPGKGLEWVGRIRSKYNNYATYYADSVKDRFTISRDDSKNTLYLQMNSLKTEDTAVYYCTRHGNFGNSYVSWFAYWGQGTTVTVSSGGGGSGGGGSGGGGSQAVVTQEPSLTVSPGGTVTLTCRSSTGAVTTSNYANWVQQKPGQAPRGLIGGTNKRAPGVPARFSGSLLGGKAALTLSGAQPEDEAEYFCALWYSNLWVFGGGTKLTVLGDKTHTCPPCPAPEAAGGPSVFLFPPKPKDTLMISRTPEVTCVVVAVSHEDPEVKFNWYVDGVEVHNAKTKPREEQYNSTYRVVSVLTVLHQDWLNGKEYKCKVSNKALAAPIEKTISKAKGQPREPQVYTLPPSRDELTKNQVSLTCLVKGFYPSDIAVEWESNGQPENNYKTTPPVLDSDGSFFLYSKLTVDKSRWQQGNVFSCSVMHEALHNHYTQKSLSLSPGK

SEQ ID NO: 72 - protein, 608 aa, artificial sequence
EVQLVESGGGLVQPGGSLRLSCAASESIFSSNVMGWYRQAPGKQRELVAAVGIQGLTKIGDSVKGRFTISRDNAKNSVYLQMNSLRAEDTAVYYCAAGAYVRFLQQSPDYWGQGTQVTVSSGGGGSEVQLVESGGGLVQPGGSLKLSCAASGFTFSTYAMNWVRQAPGKGLEWVGRIRSKYNNYATYYADSVKDRFTISRDDSKNTLYLQMNSLKTEDTAVYYCTRHGNFGNSYVSWFAYWGQGTTVTVSSGGGGSGGGGSGGGGSQAVVTQEPSLTVSPGGTVTLTCRSSTGAVTTSNYANWVQQKPGQAPRGLIGGTNKRAPGVPARFSGSLLGGKAALTLSGAQPEDEAEYFCALWYSNLWVFGGGTKLTVLGEPKSSDKTHTCPPCPAPEAAGGPSVFLFPPKPKDTLMISRTPEVTCVVVAVSHEDPEVKFNWYVDGVEVHNAKTKPREEQYNSTYRVVSVLTVLHQDWLNGKEYKCKVSNKALAAPIEKTISKAKGQPREPQVYTLPPCRDELTKNQVSLWCLVKGFYPSDIAVEWESNGQPENNYKTTPPVLDSDGSFFLYSKLTVDKSRWQQGNVFSCSVMHEALHNHYTQKSLSLSPGK

SEQ ID NO: 73 - protein, 232 aa, artificial sequence
EPKSSDKTHTCPPCPAPEAAGGPSVFLFPPKPKDTLMISRTPEVTCVVVAVSHEDPEVKFNWYVDGVEVHNAKTKPREEQYNSTYRVVSVLTVLHQDWLNGKEYKCKVSNKALAAPIEKTISKAKGQPREPQVYTLPPCRDELTKNQVSLWCLVKGFYPSDIAVEWESNGQPENNYKTTPPVLDSDGSFFLYSKLTVDKSRWQQGNVFSCSVMHEALHNHYTQKSLSLSPGK

SEQ ID NO: 74 - protein, 232 aa, artificial sequence
EPKSCDKTHTCPPCPAPEAAGGPSVFLFPPKPKDTLMISRTPEVTCVVVAVSHEDPEVKFNWYVDGVEVHNAKTKPREEQYNSTYRVVSVLTVLHQDWLNGKEYKCKVSNKALAAPIEKTISKAKGQPREPQVCTLPPSRDELTKNQVSLSCAVKGFYPSDIAVEWESNGQPENNYKTTPPVLDSDGSFFLVSKLTVDKSRWQQGNVFSCSVMHEALHNHYTQKSLSLSPGK

SEQ ID NO: 75 - protein, 8 aa, artificial sequence
ETIFSSNV

SEQ ID NO: 76 - protein, 705 aa, artificial sequence
EVQLVESGGGLVQPGGSLRLSCAASGFSLSSSYWISWVRQAPGKGLEWIGSIDSGSVGITYYATWVKGRFTISRDNSKNTLYLQMNSLRAEDTAVYYCARHGDNWALDLWGQGTLVTVLEDLKNVFPPEVAVFEPSEAEISHTQKATLVCLATGFYPDHVELSWWVNGKEVHSGVCTDPQPLKEQPALQDSRYALSSRLRVSATFWQNPRNHFRCQVQFYGLSENDEWTQDRAKPVTQIVSAEAWGRGGGGSGGGGSQVQLVQSGAEVKKPGSSVKVSCKASGFAFTDYYIHWVRQAPGQGLEWMGWISPGNVNTKYNENFKGRVTITADKSTSTAYMELSSLRSEDTAVYYCARDGYSLYYFDYWGQGTLVTVSSASTKGPSVFPLAPSSKSTSGGTAALGCLVKDYFPEPVTVSWNSGALTSGVHTFPAVLQSSGLYSLSSVVTVPSSSLGTQTYICNVNHKPSNTKVDKRVEPKSCDKTHTCPPCPAPEAAGGPSVFLFPPKPKDTLMISRTPEVTCVVVDVSHEDPEVKFNWYVDGVEVHNAKTKPREEQYNSTYRVVSVLTVLHQDWLNGKEYKCKVSNKALPAPIEKTISKAKGQPREPQVYTLPPCREEMTKNQVSLWCLVKGFYPSDIAVEWESNGQPENNYKTTPPVLDSDGSFFLYSKLTVDKSRWQQGNVFSCSVMHEALHNHYTQKSLSLSPG

SEQ ID NO: 77 - protein, 475 aa, artificial sequence
EVQLVESGGGLVQPGGSLRLSCAASGFSLSSSYWISWVRQAPGKGLEWIGSIDSGSVGITYYATWVKGRFTISRDNSKNTLYLQMNSLRAEDTAVYYCARHGDNWALDLWGQGTLVTVLEDLKNVFPPEVAVFEPSEAEISHTQKATLVCLATGFYPDHVELSWWVNGKEVHSGVCTDPQPLKEQPALQDSRYALSSRLRVSATFWQNPRNHFRCQVQFYGLSENDEWTQDRAKPVTQIVSAEAWGRASDKTHTCPPCPAPEAAGGPSVFLFPPKPKDTLMISRTPEVTCVVVDVSHEDPEVKFNWYVDGVEVHNAKTKPREEQYNSTYRVVSVLTVLHQDWLNGKEYKCKVSNKALPAPIEKTISKAKGQPREPQVCTLPPSREEMTKNQVSLSCAVKGFYPSDIAVEWESNGQPENNYKTTPPVLDSDGSFFLVSKLTVDKSRWQQGNVFSCSVMHEALHNHYTQKSLSLSPG

SEQ ID NO: 78 - protein, 219 aa, artificial sequence
DIVMTQSPDSLAVSLGERATINCKSSQSLLNSRTRKNYLAWYQQKPGQPPKLLIYWASTRQSGVPDRFSGSGSGTDFTLTISSLQAEDVAVYYCTQSHTLRTFGGGTKVEIKRTVAAPSVFIFPPSDEQLKSGTASVVCLLNNFYPREAKVQWKVDNALQSGNSQESVTEQDSKDSTYSLSSTLTLSKADYEKHKVYACEVTHQGLSSPVTKSFNRGEC

SEQ ID NO: 79 - protein, 205 aa, artificial sequence
DIQMTQSPSTLSASVGDRVTITCRASQSISSWLAWYQQKPGKAPKLLIYKASTLASGVPSRFSGSGSGTEFTLTISSLQPDDFATYYCQHGYIRGDLDNVFGGGTKVEIKPDIQNPDPAVYQLRDSKSSDKSVCLFTDFDSQTQVSQSKDSDVYITDKCVLDMRSMDFKSNSAVAWSQKSDFACANAFQNSIIPEDTFFPAPESS

SEQ ID NO: 80-81 - skipped (2 entries)

SEQ ID NO: 82 - protein, 5 aa, artificial sequence
  REPEAT 1..5: note = Repeated for n times, wherein n is an integer equal to or more than 1, for exmaple, n is a integer selected from 2, 3, 4, 5, 6, 7, 8, 9, 10.
GSGGS

SEQ ID NO: 83 - protein, 5 aa, artificial sequence
  REPEAT 1..5: note = Repeated for n times, wherein n is an integer equal to or more than 1, for exmaple, n is a integer selected from 2, 3, 4, 5, 6, 7, 8, 9, 10.
GGGGS

SEQ ID NO: 84 - protein, 4 aa, artificial sequence
  REPEAT 1..4: note = Repeated for n times, wherein n is an integer equal to or more than 1, for exmaple, n is a integer selected from 2, 3, 4, 5, 6, 7, 8, 9, 10.
GGGS

SEQ ID NO: 85 - protein, 6 aa, artificial sequence
  REPEAT 1..5: note = Repeated for n times, wherein n is an integer equal to or more than 1, for exmaple, n is a integer selected from 2, 3, 4, 5, 6, 7, 8, 9, 10.
GGGGSG

SEQ ID NO: 86 - protein, 5 aa, artificial sequence
  REPEAT 1..5: note = Repeated for n times, wherein n=1, 2, 3, 4 or 5; preferably n=3 or 4, more preferably n=3
GGGGS

SEQ ID NO: 87 - protein, 228 aa, artificial sequence
EVQLVESGGGLVQPGGSLKLSCAASGFTFSTYAMNWVRQAPGKGLEWVGRIRSKYNNYATYYADSVKDRFTISRDDSKNTLYLQMNSLKTEDTAVYYCTRHGNFGNSYVSWFAYWGQGTTVTVSSASTKGPSVFPLAPSSKSTSGGTAALGCLVKDYFPEPVTVSWNSGALTSGVHTFPAVLQSSGLYSLSSVVTVPSSSLGTQTYICNVNHKPSNTKVDKKVEPKSC